European Patent Application EP 4 640 698 A2, published October 29, 2025. Title: ANTIBODIES TO MUCIN-16 AND METHODS OF USE THEREOF. Applicant: MEMORIAL SLOAN KETTERING CANCER CENTER. Application JP 2024-173015, filed October 2, 2024. The sequence listing filed with the application follows.

SEQUENCE LISTING (33 sequences)

SEQ ID NO: 1 - protein, 14507 aa, Homo sapiens
MLKPSGLPGSSSPTRSLMTGSRSTKATPEMDSGLTGATLSPKTSTGAIVVTEHTLPFTSPDKTLASPTSSVVGRTTQSLGVMSSALPESTSRGMTHSEQRTSPSLSPQVNGTPSRNYPATSMVSGLSSPRTRTSSTEGNFTKEASTYTLTVETTSGPVTEKYTVPTETSTTEGDSTETPWDTRYIPVKITSPMKTFADSTASKENAPVSMTPAETTVTDSHTPGRTNPSFGTLYSSFLDLSPKGTPNSRGETSLELILSTTGYPFSSPEPGSAGHSRISTSAPLSSSASVLDNKISETSIFSGQSLTSPLSPGVPEARASTMPNSAIPFSMTLSNAETSAERVRSTISSLGTPSISTKQTAETILTFHAFAETMDIPSTHIAKTLASEWLGSPGTLGGTSTSALTTTSPSTTLVSEETNTHHSTSGKETEGTLNTSMTPLETSAPGEESEMTATLVPTLGFTTLDSKIRSPSQVSSSHPTRELRTTGSTSGRQSSSTAAHGSSDILRATTSSTSKASSWTSESTAQQFSEPQHTQWVETSPSMKTERPPASTSVAAPITTSVPSVVSGFTTLKTSSTKGIWLEETSADTLIGESTAGPTTHQFAVPTGISMTGGSSTRGSQGTTHLLTRATASSETSADLTLATNGVPVSVSPAVSKTAAGSSPPGGTKPSYTMVSSVIPETSSLQSSAFREGTSLGLTPLNTRHPFSSPEPDSAGHTKISTSIPLLSSASVLEDKVSATSTFSHHKATSSITTGTPEISTKTKPSSAVLSSMTLSNAATSPERVRNATSPLTHPSPSGEETAGSVLTLSTSAETTDSPNIHPTGTLTSESSESPSTLSLPSVSGVKTTFSSSTPSTHLFTSGEETEETSNPSVSQPETSVSRVRTTLASTSVPTPVFPTMDTWPTRSAQFSSSHLVSELRATSSTSVTNSTGSALPKISHLTGTATMSQTNRDTFNDSAAPQSTTWPETSPRFKTGLPSATTTVSTSATSLSATVMVSKFTSPATSSMEATSIREPSTTILTTETTNGPGSMAVASTNIPIGKGYITEGRLDTSHLPIGTTASSETSMDFTMAKESVSMSVSPSQSMDAAGSSTPGRTSQFVDTFSDDVYHLTSREITIPRDGTSSALTPQMTATHPPSPDPGSARSTWLGILSSSPSSPTPKVTMSSTFSTQRVTTSMIMDTVETSRWNMPNLPSTTSLTPSNIPTSGAIGKSTLVPLDTPSPATSLEASEGGLPTLSTYPESTNTPSIHLGAHASSESPSTIKLTMASVVKPGSYTPLTFPSIETHIHVSTARMAYSSGSSPEMTAPGETNTGSTWDPTTYITTTDPKDTSSAQVSTPHSVRTLRTTENHPKTESATPAAYSGSPKISSSPNLTSPATKAWTITDTTEHSTQLHYTKLAEKSSGFETQSAPGPVSVVIPTSPTIGSSTLELTSDVPGEPLVLAPSEQTTITLPMATWLSTSLTEEMASTDLDISSPSSPMSTFAIFPPMSTPSHELSKSEADTSAIRNTDSTTLDQHLGIRSLGRTGDLTTVPITPLTTTWTSVIEHSTQAQDTLSATMSPTHVTQSLKDQTSIPASASPSHLTEVYPELGTQGRSSSEATTFWKPSTDTLSREIETGPTNIQSTPPMDNTTTGSSSSGVTLGIAHLPIGTSSPAETSTNMALERRSSTATVSMAGTMGLLVTSAPGRSISQSLGRVSSVLSESTTEGVTDSSKGSSPRLNTQGNTALSSSLEPSYAEGSQMSTSIPLTSSPTTPDVEFIGGSTFWTKEVTTVMTSDISKSSARTESSSATLMSTALGSTENTGKEKLRTASMDLPSPTPSMEVTPWISLTLSNAPNTTDSLDLSHGVHTSSAGTLATDRSLNTGVTRASRLENGSDTSSKSLSMGNSTHTSMTYTEKSEVSSSIHPRPETSAPGAETTLTSTPGNRAISLTLPFSSIPVEEVISTGITSGPDINSAPMTHSPITPPTIVWTSTGTIEQSTQPLHAVSSEKVSVQTQSTPYVNSVAVSASPTHENSVSSGSSTSSPYSSASLESLDSTISRRNAITSWLWDLTTSLPTTTWPSTSLSEALSSGHSGVSNPSSTTTEFPLFSAASTSAAKQRNPETETHGPQNTAASTLNTDASSVTGLSETPVGASISSEVPLPMAITSRSDVSGLTSESTANPSLGTASSAGTKLTRTISLPTSESLVSFRMNKDPWTVSIPLGSHPTTNTETSIPVNSAGPPGLSTVASDVIDTPSDGAESIPTVSFSPSPDTEVTTISHFPEKTTHSFRTISSLTHELTSRVTPIPGDWMSSAMSTKPTGASPSITLGERRTITSAAPTTSPIVLTASFTETSTVSLDNETTVKTSDILDARKTNELPSDSSSSSDLINTSIASSTMDVTKTASISPTSISGMTASSSPSLFSSDRPQVPTSTTETNTATSPSVSSNTYSLDGGSNVGGTPSTLPPFTITHPVETSSALLAWSRPVRTFSTMVSTDTASGENPTSSNSVVTSVPAPGTWTSVGSTTDLPAMGFLKTSPAGEAHSLLASTIEPATAFTPHLSAAVVTGSSATSEASLLTTSESKAIHSSPQTPTTPTSGANWETSATPESLLVVTETSDTTLTSKILVTDTILFSTVSTPPSKFPSTGTLSGASFPTLLPDTPAIPLTATEPTSSLATSFDSTPLVTIASDSLGTVPETTLTMSETSNGDALVLKTVSNPDRSIPGITIQGVTESPLHPSSTSPSKIVAPRNTTYEGSITVALSTLPAGTTGSLVFSQSSENSETTALVDSSAGLERASVMPLTTGSQGMASSGGIRSGSTHSTGTKTFSSLPLTMNPGEVTAMSEITTNRLTATQSTAPKGIPVKPTSAESGLLTPVSASSSPSKAFASLTTAPPTWGIPQSTLTFEFSEVPSLDTKSASLPTPGQSLNTIPDSDASTASSSLSKSPEKNPRARMMTSTKAISASSFQSTGFTETPEGSASPSMAGHEPRVPTSGTGDPRYASESMSYPDPSKASSAMTSTSLASKLTTLFSTGQAARSGSSSSPISLSTEKETSFLSPTASTSRKTSLFLGPSMARQPNILVHLQTSALTLSPTSTLNMSQEEPPELTSSQTIAEEEGTTAETQTLTFTPSETPTSLLPVSSPTEPTARRKSSPETWASSISVPAKTSLVETTDGTLVTTIKMSSQAAQGNSTWPAPAEETGSSPAGTSPGSPEMSTTLKIMSSKEPSISPEIRSTVRNSPWKTPETTVPMETTVEPVTLQSTALGSGSTSISHLPTGTTSPTKSPTENMLATERVSLSPSPPEAWTNLYSGTPGGTRQSLATMSSVSLESPTARSITGTGQQSSPELVSKTTGMEFSMWHGSTGGTTGDTHVSLSTSSNILEDPVTSPNSVSSLTDKSKHKTETWVSTTAIPSTVLNNKIMAAEQQTSRSVDEAYSSTSSWSDQTSGSDITLGASPDVTNTLYITSTAQTTSLVSLPSGDQGITSLTNPSGGKTSSASSVTSPSIGLETLRANVSAVKSDIAPTAGHLSQTSSPAEVSILDVTTAPTPGISTTITTMGTNSISTTTPNPEVGMSTMDSTPATERRTTSTEHPSTWSSTAASDSWTVTDMTSNLKVARSPGTISTMHTTSFLASSTELDSMSTPHGRITVIGTSLVTPSSDASAVKTETSTSERTLSPSDTTASTPISTFSRVQRMSISVPDILSTSWTPSSTEAEDVPVSMVSTDHASTKTDPNTPLSTFLFDSLSTLDWDTGRSLSSATATTSAPQGATTPQELTLETMISPATSQLPFSIGHITSAVTPAAMARSSGVTFSRPDPTSKKAEQTSTQLPTTTSAHPGQVPRSAATTLDVIPHTAKTPDATFQRQGQTALTTEARATSDSWNEKEKSTPSAPWITEMMNSVSEDTIKEVTSSSSVLRTLNTLDINLESGTTSSPSWKSSPYERIAPSESTTDKEAIHPSTNTVETTGWVTSSEHASHSTIPAHSASSKLTSPVVTTSTREQAIVSMSTTTWPESTRARTEPNSFLTIELRDVSPYMDTSSTTQTSIISSPGSTAITKGPRTEITSSKRISSSFLAQSMRSSDSPSEAITRLSNFPAMTESGGMILAMQTSPPGATSLSAPTLDTSATASWTGTPLATTQRFTYSEKTTLFSKGPEDTSQPSPPSVEETSSSSSLVPIHATTSPSNILLTSQGHSPSSTPPVTSVFLSETSGLGKTTDMSRISLEPGTSLPPNLSSTAGEALSTYEASRDTKAIHHSADTAVTNMEATSSEYSPIPGHTKPSKATSPLVTSHIMGDITSSTSVFGSSETTEIETVSSVNQGLQERSTSQVASSATETSTVITHVSSGDATTHVTKTQATFSSGTSISSPHQFITSTNTFTDVSTNPSTSLIMTESSGVTITTQTGPTGAATQGPYLLDTSTMPYLTETPLAVTPDFMQSEKTTLISKGPKDVSWTSPPSVAETSYPSSLTPFLVTTIPPATSTLQGQHTSSPVSATSVLTSGLVKTTDMLNTSMEPVTNSPQNLNNPSNEILATLAATTDIETIHPSINKAVTNMGTASSAHVLHSTLPVSSEPSTATSPMVPASSMGDALASISIPGSETTDIEGEPTSSLTAGRKENSTLQEMNSTTESNIILSNVSVGAITEATKMEVPSFDATFIPTPAQSTKFPDIFSVASSRLSNSPPMTISTHMTTTQTGSSGATSKIPLALDTSTLETSAGTPSVVTEGFAHSKITTAMNNDVKDVSQTNPPFQDEASSPSSQAPVLVTTLPSSVAFTPQWHSTSSPVSMSSVLTSSLVKTAGKVDTSLETVTSSPQSMSNTLDDISVTSAATTDIETTHPSINTVVTNVGTTGSAFESHSTVSAYPEPSKVTSPNVTTSTMEDTTISRSIPKSSKTTRTETETTSSLTPKLRETSISQEITSSTETSTVPYKELTGATTEVSRTDVTSSSSTSFPGPDQSTVSLDISTETNTRLSTSPIMTESAEITITTQTGPHGATSQDTFTMDPSNTTPQAGIHSAMTHGFSQLDVTTLMSRIPQDVSWTSPPSVDKTSSPSSFLSSPAMTTPSLISSTLPEDKLSSPMTSLLTSGLVKITDILRTRLEPVTSSLPNFSSTSDKILATSKDSKDTKEIFPSINTEETNVKANNSGHESHSPALADSETPKATTQMVITTTVGDPAPSTSMPVHGSSETTNIKREPTYFLTPRLRETSTSQESSFPTDTSFLLSKVPTGTITEVSSTGVNSSSKISTPDHDKSTVPPDTFTGEIPRVFTSSIKTKSAEMTITTQASPPESASHSTLPLDTSTTLSQGGTHSTVTQGFPYSEVTTLMGMGPGNVSWMTTPPVEETSSVSSLMSSPAMTSPSPVSSTSPQSIPSSPLPVTALPTSVLVTTTDVLGTTSPESVTSSPPNLSSITHERPATYKDTAHTEAAMHHSTNTAVTNVGTSGSGHKSQSSVLADSETSKATPLMSTTSTLGDTSVSTSTPNISQTNQIQTEPTASLSPRLRESSTSEKTSSTTETNTAFSYVPTGAITQASRTEISSSRTSISDLDRPTIAPDISTGMITRLFTSPIMTKSAEMTVTTQTTTPGATSQGILPWDTSTTLFQGGTHSTVSQGFPHSEITTLRSRTPGDVSWMTTPPVEETSSGFSLMSPSMTSPSPVSSTSPESIPSSPLPVTALLTSVLVTTTNVLGTTSPEPVTSSPPNLSSPTQERLTTYKDTAHTEAMHASMHTNTAVANVGTSISGHESQSSVPADSHTSKATSPMGITFAMGDTSVSTSTPAFFETRIQTESTSSLIPGLRDTRTSEEINTVTETSTVLSEVPTTTTTEVSRTEVITSSRTTISGPDHSKMSPYISTETITRLSTFPFVTGSTEMAITNQTGPIGTISQATLTLDTSSTASWEGTHSPVTQRFPHSEETTTMSRSTKGVSWQSPPSVEETSSPSSPVPLPAITSHSSLYSAVSGSSPTSALPVTSLLTSGRRKTIDMLDTHSELVTSSLPSASSFSGEILTSEASTNTETIHFSENTAETNMGTTNSMHKLHSSVSIHSQPSGHTPPKVTGSMMEDAIVSTSTPGSPETKNVDRDSTSPLTPELKEDSTALVMNSTTESNTVFSSVSLDAATEVSRAEVTYYDPTFMPASAQSTKSPDISPEASSSHSNSPPLTISTHKTIATQTGPSGVTSLGQLTLDTSTIATSAGTPSARTQDFVDSETTSVMNNDLNDVLKTSPFSAEEANSLSSQAPLLVTTSPSPVTSTLQEHSTSSLVSVTSVPTPTLAKITDMDTNLEPVTRSPQNLRNTLATSEATTDTHTMHPSINTAVANVGTTSSPNEFYFTVSPDSDPYKATSAVVITSTSGDSIVSTSMPRSSAMKKIESETTFSLIFRLRETSTSQKIGSSSDTSTVFDKAFTAATTEVSRTELTSSSRTSIQGTEKPTMSPDTSTRSVTMLSTFAGLTKSEERTIATQTGPHRATSQGTLTWDTSITTSQAGTHSAMTHGFSQLDLSTLTSRVPEYISGTSPPSVEKTSSSSSLLSLPAITSPSPVPTTLPESRPSSPVHLTSLPTSGLVKTTDMLASVASLPPNLGSTSHKIPTTSEDIKDTEKMYPSTNIAVTNVGTTTSEKESYSSVPAYSEPPKVTSPMVTSFNIRDTIVSTSMPGSSEITRIEMESTFSLAHGLKGTSTSQDPIVSTEKSAVLHKLTTGATETSRTEVASSRRTSIPGPDHSTESPDISTEVIPSLPISLGITESSNMTIITRTGPPLGSTSQGTFTLDTPTTSSRAGTHSMATQEFPHSEMTTVMNKDPEILSWTIPPSIEKTSFSSSLMPSPAMTSPPVSSTLPKTIHTTPSPMTSLLTPSLVMTTDTLGTSPEPTTSSPPNLSSTSHEILTTDEDTTAIEAMHPSTSTAATNVETTSSGHGSQSSVLADSEKTKATAPMDTTSTMGHTTVSTSMSVSSETTKIKRESTYSLTPGLRETSISQNASFSTDTSIVLSEVPTGTTAEVSRTEVTSSGRTSIPGPSQSTVLPEISTRTMTRLFASPTMTESAEMTIPTQTGPSGSTSQDTLTLDTSTTKSQAKTHSTLTQRFPHSEMTTLMSRGPGDMSWQSSPSLENPSSLPSLLSLPATTSPPPISSTLPVTISSSPLPVTSLLTSSPVTTTDMLHTSPELVTSSPPKLSHTSDERLTTGKDTTNTEAVHPSTNTAASNVEIPSSGHESPSSALADSETSKATSPMFITSTQEDTTVAISTPHFLETSRIQKESISSLSPKLRETGSSVETSSAIETSAVLSEVSIGATTEISRTEVTSSSRTSISGSAESTMLPEISTTRKIIKFPTSPILAESSEMTIKTQTSPPGSTSESTFTLDTSTTPSLVITHSTMTQRLPHSEITTLVSRGAGDVPRPSSLPVEETSPPSSQLSLSAMISPSPVSSTLPASSHSSSASVTSLLTPGQVKTTEVLDASAEPETSSPPSLSSTSVEILATSEVTTDTEKIHPFSNTAVTKVGTSSSGHESPSSVLPDSETTKATSAMGTISIMGDTSVSTLTPALSNTRKIQSEPASSLTTRLRETSTSEETSLATEANTVLSKVSTGATTEVSRTEAISFSRTSMSGPEQSTMSQDISIGTIPRISASSVLTESAKMTITTQTGPSESTLESTLNLNTATTPSWVETHSIVIQGFPHPEMTTSMGRGPGGVSWPSPPFVKETSPPSSPLSLPAVTSPHPVSTTFLAHIPPSPLPVTSLLTSGPATTTDILGTSTEPGTSSSSSLSTTSHERLTTYKDTAHTEAVHPSTNTGGTNVATTSSGYKSQSSVLADSSPMCTTSTMGDTSVLTSTPAFLETRRIQTELASSLTPGLRESSGSEGTSSGTKMSTVLSKVPTGATTEISKEDVTSIPGPAQSTISPDISTRTVSWFSTSPVMTESAEITMNTHTSPLGATTQGTSTLDTSSTTSLTMTHSTISQGFSHSQMSTLMRRGPEDVSWMSPPLLEKTRPSFSLMSSPATTSPSPVSSTLPESISSSPLPVTSLLTSGLAKTTDMLHKSSEPVTNSPANLSSTSVEILATSEVTTDTEKTHPSSNRTVTDVGTSSSGHESTSFVLADSQTSKVTSPMVITSTMEDTSVSTSTPGFFETSRIQTEPTSSLTLGLRKTSSSEGTSLATEMSTVLSGVPTGATAEVSRTEVTSSSRTSISGFAQLTVSPETSTETITRLPTSSIMTESAEMMIKTQTDPPGSTPESTHTVDISTTPNWVETHSTVTQRFSHSEMTTLVSRSPGDMLWPSQSSVEETSSASSLLSLPATTSPSPVSSTLVEDFPSASLPVTSLLNPGLVITTDRMGISREPGTSSTSNLSSTSHERLTTLEDTVDTEDMQPSTHTAVTNVRTSISGHESQSSVLSDSETPKATSPMGTTYTMGETSVSISTSDFFETSRIQIEPTSSLTSGLRETSSSERISSATEGSTVLSEVPSGATTEVSRTEVISSRGTSMSGPDQFTISPDISTEAITRLSTSPIMTESAESAITIETGSPGATSEGTLTLDTSTTTFWSGTHSTASPGFSHSEMTTLMSRTPGDVPWPSLPSVEEASSVSSSLSSPAMTSTSFFSTLPESISSSPHPVTALLTLGPVKTTDMLRTSSEPETSSPPNLSSTSAEILATSEVTKDREKIHPSSNTPVVNVGTVIYKHLSPSSVLADLVTTKPTSPMATTSTLGNTSVSTSTPAFPETMMTQPTSSLTSGLREISTSQETSSATERSASLSGMPTGATTKVSRTEALSLGRTSTPGPAQSTISPEISTETITRISTPLTTTGSAEMTITPKTGHSGASSQGTFTLDTSSRASWPGTHSAATHRSPHSGMTTPMSRGPEDVSWPSRPSVEKTSPPSSLVSLSAVTSPSPLYSTPSESSHSSPLRVTSLFTPVMMKTTDMLDTSLEPVTTSPPSMNITSDESLATSKATMETEAIQLSENTAVTQMGTISARQEFYSSYPGLPEPSKVTSPVVTSSTIKDIVSTTIPASSEITRIEMESTSTLTPTPRETSTSQEIHSATKPSTVPYKALTSATIEDSMTQVMSSSRGPSPDQSTMSQDISTEVITRLSTSPIKTESTEMTITTQTGSPGATSRGTLTLDTSTTFMSGTHSTASQGFSHSQMTALMSRTPGDVPWLSHPSVEEASSASFSLSSPVMTSSSPVSSTLPDSIHSSSLPVTSLLTSGLVKTTELLGTSSEPETSSPPNLSSTSAEILAITEVTTDTEKLEMTNVVTSGYTHESPSSVLADSVTTKATSSMGITYPTGDTNVLTSTPAFSDTSRIQTKSKLSLTPGLMETSISEETSSATEKSTVLSSVPTGATTEVSRTEAISSSRTSIPGPAQSTMSSDTSMETITRISTPLTRKESTDMAITPKTGPSGATSQGTFTLDSSSTASWPGTHSATTQRFPQSVVTTPMSRGPEDVSWPSPLSVEKNSPPSSLVSSSSVTSPSPLYSTPSGSSHSSPVPVTSLFTSIMMKATDMLDASLEPETTSAPNMNITSDESLAASKATTETEAIHVFENTAASHVETTSATEELYSSSPGFSEPTKVISPVVTSSSIRDNMVSTTMPGSSGITRIEIESMSSLTPGLRETRTSQDITSSTETSTVLYKMPSGATPEVSRTEVMPSSRTSIPGPAQSTMSLDISDEVVTRLSTSPIMTESAEITITTQTGYSLATSQVTLPLGTSMTFLSGTHSTMSQGLSHSEMTNLMSRGPESLSWTSPRFVETTRSSSSLTSLPLTTSLSPVSSTLLDSSPSSPLPVTSLILPGLVKTTEVLDTSSEPKTSSSPNLSSTSVEIPATSEIMTDTEKIHPSSNTAVAKVRTSSSVHESHSSVLADSETTITIPSMGITSAVDDTTVFTSNPAFSETRRIPTEPTFSLTPGFRETSTSEETTSITETSAVLYGVPTSATTEVSMTEIMSSNRIHIPDSDQSTMSPDIITEVITRLSSSSMMSESTQMTITTQKSSPGATAQSTLTLATTTAPLARTHSTVPPRFLHSEMTTLMSRSPENPSWKSSLFVEKTSSSSSLLSLPVTTSPSVSSTLPQSIPSSSFSVTSLLTPGMVKTTDTSTEPGTSLSPNLSGTSVEILAASEVTTDTEKIHPSSSMAVTNVGTTSSGHELYSSVSIHSEPSKATYPVGTPSSMAETSISTSMPANFETTGFEAEPFSHLTSGFRKTNMSLDTSSVTPTNTPSSPGSTHLLQSSKTDFTSSAKTSSPDWPPASQYTEIPVDIITPFNASPSITESTGITSFPESRFTMSVTESTHHLSTDLLPSAETISTGTVMPSLSEAMTSFATTGVPRAISGSGSPFSRTESGPGDATLSTIAESLPSSTPVPFSSSTFTTTDSSTIPALHEITSSSATPYRVDTSLGTESSTTEGRLVMVSTLDTSSQPGRTSSSPILDTRMTESVELGTVTSAYQVPSLSTRLTRTDGIMEHITKIPNEAAHRGTIRPVKGPQTSTSPASPKGLHTGGTKRMETTTTALKTTTTALKTTSRATLTTSVYTPTLGTLTPLNASMQMASTIPTEMMITTPYVFPDVPETTSSLATSLGAETSTALPRTTPSVFNRESETTASLVSRSGAERSPVIQTLDVSSSEPDTTASWVIHPAETIPTVSKTTPNFFHSELDTVSSTATSHGADVSSAIPTNISPSELDALTPLVTISGTDTSTTFPTLTKSPHETETRTTWLTHPAETSSTIPRTIPNFSHHESDATPSIATSPGAETSSAIPIMTVSPGAEDLVTSQVTSSGTDRNMTIPTLTLSPGEPKTIASLVTHPEAQTSSAIPTSTISPAVSRLVTSMVTSLAAKTSTTNRALTNSPGEPATTVSLVTHPAQTSPTVPWTTSIFFHSKSDTTPSMTTSHGAESSSAVPTPTVSTEVPGVVTPLVTSSRAVISTTIPILTLSPGEPETTPSMATSHGEEASSAIPTPTVSPGVPGVVTSLVTSSRAVTSTTIPILTFSLGEPETTPSMATSHGTEAGSAVPTVLPEVPGMVTSLVASSRAVTSTTLPTLTLSPGEPETTPSMATSHGAEASSTVPTVSPEVPGVVTSLVTSSSGVNSTSIPTLILSPGELETTPSMATSHGAEASSAVPTPTVSPGVSGVVTPLVTSSRAVTSTTIPILTLSSSEPETTPSMATSHGVEASSAVLTVSPEVPGMVTSLVTSSRAVTSTTIPTLTISSDEPETTTSLVTHSEAKMISAIPTLAVSPTVQGLVTSLVTSSGSETSAFSNLTVASSQPETIDSWVAHPGTEASSVVPTLTVSTGEPFTNISLVTHPAESSSTLPRTTSRFSHSELDTMPSTVTSPEAESSSAISTTISPGIPGVLTSLVTSSGRDISATFPTVPESPHESEATASWVTHPAVTSTTVPRTTPNYSHSEPDTTPSIATSPGAEATSDFPTITVSPDVPDMVTSQVTSSGTDTSITIPTLTLSSGEPETTTSFITYSETHTSSAIPTLPVSPGASKMLTSLVISSGTDSTTTFPTLTETPYEPETTAIQLIHPAETNTMVPRTTPKFSHSKSDTTLPVAITSPGPEASSAVSTTTISPDMSDLVTSLVPSSGTDTSTTFPTLSETPYEPETTATWLTHPAETSTTVSGTIPNFSHRGSDTAPSMVTSPGVDTRSGVPTTTIPPSIPGVVTSQVTSSATDTSTAIPTLTPSPGEPETTASSATHPGTQTGFTVPIRTVPSSEPDTMASWVTHPPQTSTPVSRTTSSFSHSSPDATPVMATSPRTEASSAVLTTISPGAPEMVTSQITSSGAATSTTVPTLTHSPGMPETTALLSTHPRTETSKTFPASTVFPQVSETTASLTIRPGAETSTALPTQTTSSLFTLLVTGTSRVDLSPTASPGVSAKTAPLSTHPGTETSTMIPTSTLSLGLLETTGLLATSSSAETSTSTLTLTVSPAVSGLSSASITTDKPQTVTSWNTETSPSVTSVGPPEFSRTVTGTTMTLIPSEMPTPPKTSHGEGVSPTTILRTTMVEATNLATTGSSPTVAKTTTTFNTLAGSLFTPLTTPGMSTLASESVTSRTSYNHRSWISTTSSYNRRYWTPATSTPVTSTFSPGISTSSIPSSTAATVPFMVPFTLNFTITNLQYEEDMRHPGSRKFNATERELQGLLKPLFRNSSLEYLYSGCRLASLRPEKDSSATAVDAICTHRPDPEDLGLDRERLYWELSNLTNGIQELGPYTLDRNSLYVNGFTHRSSMPTTSTPGTSTVDVGTSGTPSSSPSPTTAGPLLMPFTLNFTITNLQYEEDMRRTGSRKFNTMESVLQGLLKPLFKNTSVGPLYSGCRLTLLRPEKDGAATGVDAICTHRLDPKSPGLNREQLYWELSKLTNDIEELGPYTLDRNSLYVNGFTHQSSVSTTSTPGTSTVDLRTSGTPSSLSSPTIMAAGPLLVPFTLNFTITNLQYGEDMGHPGSRKFNTTERVLQGLLGPIFKNTSVGPLYSGCRLTSLRSEKDGAATGVDAICIHHLDPKSPGLNRERLYWELSQLTNGIKELGPYTLDRNSLYVNGFTHRTSVPTSSTPGTSTVDLGTSGTPFSLPSPATAGPLLVLFTLNFTITNLKYEEDMHRPGSRKFNTTERVLQTLLGPMFKNTSVGLLYSGCRLTLLRSEKDGAATGVDAICTHRLDPKSPGVDREQLYWELSQLTNGIKELGPYTLDRNSLYVNGFTHWIPVPTSSTPGTSTVDLGSGTPSSLPSPTTAGPLLVPFTLNFTITNLKYEEDMHCPGSRKFNTTERVLQSLLGPMFKNTSVGPLYSGCRLTLLRSEKDGAATGVDAICTHRLDPKSPGVDREQLYWELSQLTNGIKELGPYTLDRNSLYVNGFTHQTSAPNTSTPGTSTVDLGTSGTPSSLPSPTSAGPLLVPFTLNFTITNLQYEEDMHHPGSRKFNTTERVLQGLLGPMFKNTSVGLLYSGCRLTLLRPEKNGAATGMDAICSHRLDPKSPGLNREQLYWELSQLTHGIKELGPYTLDRNSLYVNGFTHRSSVAPTSTPGTSTVDLGTSGTPSSLPSPTTAVPLLVPFTLNFTITNLQYGEDMRHPGSRKFNTTERVLQGLLGPLFKNSSVGPLYSGCRLISLRSEKDGAATGVDAICTHHLNPQSPGLDREQLYWQLSQMTNGIKELGPYTLDRNSLYVNGFTHRSSGLTTSTPWTSTVDLGTSGTPSPVPSPTTTGPLLVPFTLNFTITNLQYEENMGHPGSRKFNITESVLQGLLKPLFKSTSVGPLYSGCRLTLLRPEKDGVATRVDAICTHRPDPKIPGLDRQQLYWELSQLTHSITELGPYTLDRDSLYVNGFTQRSSVPTTSTPGTFTVQPETSETPSSLPGPTATGPVLLPFTLNFTITNLQYEEDMRRPGSRKFNTTERVLQGLLMPLFKNTSVSSLYSGCRLTLLRPEKDGAATRVDAVCTHRPDPKSPGLDRERLYWKLSQLTHGITELGPYTLDRHSLYVNGFTHQSSMTTTRTPDTSTMHLATSRTPASLSGPMTASPLLVLFTINFTITNLRYEENMHHPGSRKFNTTERVLQGLLRPVFKNTSVGPLYSGCRLTLLRPKKDGAATKVDAICTYRPDPKSPGLDREQLYWELSQLTHSITELGPYTLDRDSLYVNGFTQRSSVPTTSIPGTPTVDLGTSGTPVSKPGPSAASPLLVLFTLNFTITNLRYEENMQHPGSRKFNTTERVLQGLLRSLFKSTSVGPLYSGCRLTLLRPEKDGTATGVDAICTHHPDPKSPRLDREQLYWELSQLTHNITELGPYALDNDSLFVNGFTHRSSVSTTSTPGTPTVYLGASKTPASIFGPSAASHLLILFTLNFTITNLRYEENMWPGSRKFNTTERVLQGLLRPLFKNTSVGPLYSGCRLTLLRPEKDGEATGVDAICTHRPDPTGPGLDREQLYLELSQLTHSITELGPYTLDRDSLYVNGFTHRSSVPTTSTGVVSEEPFTLNFTINNLRYMADMGQPGSLKFNITDNVMQHLLSPLFQRSSLGARYTGCRVIALRSVKNGAETRVDLLCTYLQPLSGPGLPIKQVFHELSQQTHGITRLGPYSLDKDSLYLNGYNEPGPDEPPTTPKPATTFLPPLSEATTAMGYHLKTLTLNFTISNLQYSPDMGKGSATFNSTEGVLQHLLRPLFQKSSMGPFYLGCQLISLRPEKDGAATGVDTTCTYHPDPVGPGLDIQQLYWELSQLTHGVTQLGFYVLDRDSLFINGYAPQNLSIRGEYQINFHIVNWNLSNPDPTSSEYITLLRDIQDKVTTLYKGSQLHDTFRFCLVTNLTMDSVLVTVKALFSSNLDPSLVEQVFLDKTLNASFHWLGSTYQLVDIHVTEMESSVYQPTSSSSTQHFYLNFTITNLPYSQDKAQPGTTNYQRNKRNIEDALNQLFRNSSIKSYFSDCQVSTFRSVPNRHHTGVDSLCNFSPLARRVDRVAIYEEFLRMTRNGTQLQNFTLDRSSVLVDGYSPNRNEPLTGNSDLPFWAVILIGLAGLLGVITCLICGVLVTTRRRKKEGEYNVQQQCPGYYQSHLDLEDLQ

SEQ ID NO: 2 - protein, 115 aa, synthetic construct
  REGION 1..115: note = Description of Artificial Sequence: Synthetic polypeptide
QVQLQQWGAGLLKPSETLSLTCAVYGGSFSGYYWSWIRQPPGKGLEWIGEINHSGSTNYNPSLKSRVTISVDTSKNQFSLKLSSVTAADTAVYYCARQSYITDSWGQGTLVTVSS

SEQ ID NO: 3 - protein, 108 aa, synthetic construct
  REGION 1..108: note = Description of Artificial Sequence: Synthetic polypeptide
DIQLTQSPSAVSASVGDRVTITCRASQDVSKWLAWYQQKPGKAPRLLISAASGLQSWVPSRFSGSGSGTEFTLSISSLQPEDFATYYCQQANSFPWTFGQGTKVEIKR

SEQ ID NO: 4 - protein, 8 aa, synthetic construct
  REGION 1..8: note = Description of Artificial Sequence: Synthetic peptide
GGSFSGYY

SEQ ID NO: 5 - protein, 7 aa, synthetic construct
  REGION 1..7: note = Description of Artificial Sequence: Synthetic peptide
INHSGST

SEQ ID NO: 6 - protein, 9 aa, synthetic construct
  REGION 1..9: note = Description of Artificial Sequence: Synthetic peptide
ARQSYITDS

SEQ ID NO: 7 - protein, 6 aa, synthetic construct
  REGION 1..6: note = Description of Artificial Sequence: Synthetic peptide
QDVSKW

SEQ ID NO: 8 - skipped

SEQ ID NO: 9 - protein, 9 aa, synthetic construct
  REGION 1..9: note = Description of Artificial Sequence: Synthetic peptide
QQANSFPWT

SEQ ID NO: 10 - protein, 120 aa, synthetic construct
  REGION 1..120: note = Description of Artificial Sequence: Synthetic polypeptide
QVQLQQWGAGLLKPSETLSLTCAVYGGSFSGYYWSWIRQPPGKGLEWIGEINHSGSTNYNPSLKSRIIMSVDTSKRQFSLKLRSATAADTAVYYCARWSPFSYKQMYDYWGQGTLVTVSS

SEQ ID NO: 11 - protein, 112 aa, synthetic construct
  REGION 1..112: note = Description of Artificial Sequence: Synthetic polypeptide
NFMLTQPHSVSESPGKTVTISCTRSRGSIASAYVQWYQQRPGSAPITVIYEDYERPSEIPDRFSGSIDSSSNSASLTISGLKTEDEADYYCQSYDDNDHVIFGGGTKVTVLG

SEQ ID NO: 12 - protein, 8 aa, synthetic construct
  REGION 1..8: note = Description of Artificial Sequence: Synthetic peptide
GGSFSGYY

SEQ ID NO: 13 - protein, 7 aa, synthetic construct
  REGION 1..7: note = Description of Artificial Sequence: Synthetic peptide
INHSGST

SEQ ID NO: 14 - protein, 14 aa, synthetic construct
  REGION 1..14: note = Description of Artificial Sequence: Synthetic peptide
ARWSPFSYKQMYDY

SEQ ID NO: 15 - protein, 8 aa, synthetic construct
  REGION 1..8: note = Description of Artificial Sequence: Synthetic peptide
RGSIASAY

SEQ ID NO: 16 - skipped

SEQ ID NO: 17 - protein, 10 aa, synthetic construct
  REGION 1..10: note = Description of Artificial Sequence: Synthetic peptide
QSYDDNDHVI

SEQ ID NO: 18 - protein, 20 aa, synthetic construct
  REGION 1..20: note = Description of Artificial Sequence: Synthetic peptide
METDTLLLWVLLLWVPGSTG

SEQ ID NO: 19 - protein, 244 aa, synthetic construct
  REGION 1..244: note = Description of Artificial Sequence: Synthetic polypeptide
DIQLTQSPSAVSASVGDRVTITCRASQDVSKWLAWYQQKPGKAPRLLISAASGLQSWVPSRFSGSGSGTEFTLSISSLQPEDFATYYCQQANSFPWTFGQGTKVEIKRSRGGGGSGGGGSGGGGSLEMAQVQLQQWGAGLLKPSETLSLTCAVYGGSFSGYYWSWIRQPPGKGLEWIGEINHSGSTNYNPSLKSRVTISVDTSKNQFSLKLSSVTAADTAVYYCARQSYITDSWGQGTLVTVSS

SEQ ID NO: 20 - protein, 253 aa, synthetic construct
  REGION 1..253: note = Description of Artificial Sequence: Synthetic polypeptide
NFMLTQPHSVSESPGKTVTISCTRSRGSIASAYVQWYQQRPGSAPITVIYEDYERPSEIPDRFSGSIDSSSNSASLTISGLKTEDEADYYCQSYDDNDHVIFGGGTKVTVLGSRGGGGSGGGGSGGGGSLEMAQVQLQQWGAGLLKPSETLSLTCAVYGGSFSGYYWSWIRQPPGKGLEWIGEINHSGSTNYNPSLKSRIIMSVDTSKRQFSLKLRSATAADTAVYYCARWSPFSYKQMYDYWGQGTLVTVSS

SEQ ID NO: 21 - protein, 243 aa, synthetic construct
  REGION 1..243: note = Description of Artificial Sequence: Synthetic polypeptide
DVQLVQSGAEVKKPGASVKVSCKASGYTFTRYTMHWVRQAPGQGLEWIGYINPSRGYTNYADSVKGRFTITTDKSTSTAYMELSSLRSEDTATYYCARYYDDHYCLDYWGQGTTVTVSSGEGTSTGSGGSGGSGGADDIVLTQSPATLSLSPGERATLSCRASQSVSYMNWYQQKPGKAPKRWIYDTSKVASGVPARFSGSGSGTDYSLTINSLEAEDAATYYCQQWSSNPLTFGGGTKVEIK

SEQ ID NO: 22 - protein, 520 aa, synthetic construct
  REGION 1..520: note = Description of Artificial Sequence: Synthetic polypeptide
METDTLLLWVLLLWVPGSTGDIQLTQSPSAVSASVGDRVTITCRASQDVSKWLAWYQQKPGKAPRLLISAASGLQSWVPSRFSGSGSGTEFTLSISSLQPEDFATYYCQQANSFPWTFGQGTKVEIKRSRGGGGSGGGGSGGGGSLEMAQVQLQQWGAGLLKPSETLSLTCAVYGGSFSGYYWSWIRQPPGKGLEWIGEINHSGSTNYNPSLKSRVTISVDTSKNQFSLKLSSVTAADTAVYYCARQSYITDSWGQGTLVTVSSTSGGGGSDVQLVQSGAEVKKPGASVKVSCKASGYTFTRYTMHWVRQAPGQGLEWIGYINPSRGYTNYADSVKGRFTITTDKSTSTAYMELSSLRSEDTATYYCARYYDDHYCLDYWGQGTTVTVSSGEGTSTGSGGSGGSGGADDIVLTQSPATLSLSPGERATLSCRASQSVSYMNWYQQKPGKAPKRWIYDTSKVASGVPARFSGSGSGTDYSLTINSLEAEDAATYYCQQWSSNPLTFGGGTKVEIKHHHHHH

SEQ ID NO: 23 - protein, 529 aa, synthetic construct
  REGION 1..529: note = Description of Artificial Sequence: Synthetic polypeptide
METDTLLLWVLLLWVPGSTGNFMLTQPHSVSESPGKTVTISCTRSRGSIASAYVQWYQQRPGSAPITVIYEDYERPSEIPDRFSGSIDSSSNSASLTISGLKTEDEADYYCQSYDDNDHVIFGGGTKVTVLGSRGGGGSGGGGSGGGGSLEMAQVQLQQWGAGLLKPSETLSLTCAVYGGSFSGYYWSWIRQPPGKGLEWIGEINHSGSTNYNPSLKSRIIMSVDTSKRQFSLKLRSATAADTAVYYCARWSPFSYKQMYDYWGQGTLVTVSSTSGGGGSDVQLVQSGAEVKKPGASVKVSCKASGYTFTRYTMHWVRQAPGQGLEWIGYINPSRGYTNYADSVKGRFTITTDKSTSTAYMELSSLRSEDTATYYCARYYDDHYCLDYWGQGTTVTVSSGEGTSTGSGGSGGSGGADDIVLTQSPATLSLSPGERATLSCRASQSVSYMNWYQQKPGKAPKRWIYDTSKVASGVPARFSGSGSGTDYSLTINSLEAEDAATYYCQQWSSNPLTFGGGTKVEIKHHHHHH

SEQ ID NO: 24 - protein, 344 aa, synthetic construct
  REGION 1..344: note = Description of Artificial Sequence: Synthetic polypeptide
WELSQLTHGVTQLGFYVLDRDSLFINGYAPQNLSIRGEYQINFHIVNQNLSNPDPTSSEYITLLRDIQDKVTTLYKGSQLHDTFRFCLVTNLTMDSVLVTVKALFSSNLDPSLVEQVFLDKTLNASFHQLGSTYQLVDIHVTEMESSVYQPTSSSSTQHFYLNFTITNLPYSQDKAQPGTTNYQRNKRNIEDALNQLFRNSSIKSYFSDCQVSTFRSVPNRHHTGVDSLCNFSPLARRVDRVAIYEEFLRMTRNGTQLQNFTLDRSSVLVDGYSPNRNEPLTGNSDLPFWAVILIGLAGLLGLITCLICGVLVTTRRRKKEGEYNVQQQCPGYYQSHLDLEDLQ

SEQ ID NO: 25 - protein, 114 aa, synthetic construct
  REGION 1..114: note = Description of Artificial Sequence: Synthetic polypeptide
NFSPLARRVDRVAIYEEFLRMTRNGTQLQNFTLDRSSVLVDGYSPNRNEPLTGNSDLPFWAVILIGLAGLLGLITCLICGVLVTTRRRKKEGEYNVQQQCPGYYQSHLDLEDLQ

SEQ ID NO: 26 - protein, 80 aa, synthetic construct
  REGION 1..80: note = Description of Artificial Sequence: Synthetic polypeptide
NFSPLARRVDRVAIYEEFLRMDLPFWAVILIGLAGLLGLITCLICGVLVTTRRRKKEGEYNVQQQCPGYYQSHLDLEDLQ

SEQ ID NO: 27 - protein, 86 aa, synthetic construct
  REGION 1..86: note = Description of Artificial Sequence: Synthetic polypeptide
NFSPLARRVDRVAIYEEFLRMTRNGTQLQNFTLDRSSVLVDGYSPNRNEPLTGNSDLPFWAVILIGLAGLLGLITCLICGDLEDLQ

SEQ ID NO: 28 - protein, 330 aa, synthetic construct
  REGION 1..330: note = Description of Artificial Sequence: Synthetic polypeptide
ASTKGPSVFPLAPSSKSTSGGTAALGCLVKDYFPEPVTVSWNSGALTSGVHTFPAVLQSSGLYSLSSVVTVPSSSLGTQTYICNVNHKPSNTKVDKKVEPKSCDKTHTCPPCPAPELLGGPSVFLFPPKPKDTLMISRTPEVTCVVVDVSHEDPEVKFNWYVDGVEVHNAKTKPREEQYNSTYRVVSVLTVLHQDWLNGKEYKCKVSNKALPAPIEKTISKAKGQPREPQVYTLPPSREEMTKNQVSLTCLVKGFYPSDIAVEWESNGQPENNYKTTPPVLDSDGSFFLYSKLTVDKSRWQQGNVFSCSVMHEALHNHYTQKSLSLSPGK

SEQ ID NO: 29 - protein, 327 aa, synthetic construct
  REGION 1..327: note = Description of Artificial Sequence: Synthetic polypeptide
ASTKGPSVFPLAPCSRSTSESTAALGCLVKDYFPEPVTVSWNSGALTSGVHTFPAVLQSSGLYSLSSVVTVPSSSLGTKTYTCNVDHKPSNTKVDKRVESKYGPPCPSCPAPEFLGGPSVFLFPPKPKDTLMISRTPEVTCVVVDVSQEDPEVQFNWYVDGVEVHNAKTKPREEQFNSTYRVVSVLTVLHQDWLNGKEYKCKVSNKGLPSSIEKTISKAKGQPREPQVYTLPPSQEEMTKNQVSLTCLVKGFYPSDIAVEWESNGQPENNYKTTPPVLDSDGSFFLYSRLTVDKSRWQEGNVFSCSVMHEALHNHYTQKSLSLSLGK

SEQ ID NO: 30 - protein, 105 aa, synthetic construct
  REGION 1..105: note = Description of Artificial Sequence: Synthetic polypeptide
QPKANPTVTLFPPSSEELQANKATLVCLISDFYPGAVTVAWKADGSPVKAGVETTKPSKQSNNKYAASSYLSLTPEQWKSHRSYSCQVTHEGSTVEKTVAPTECS

SEQ ID NO: 31 - protein, 114 aa, synthetic construct
  REGION 1..114: note = Description of Artificial Sequence: Synthetic polypeptide
NFSPLARRVDRVAIYEEFLRMTRNGTQLQAFTLDRSSVLVDGYSPNRNEPLTGNSDLPFWAVILIGLAGLLGLITCLICGVLVTTRRRKKEGEYNVQQQCPGYYQSHLDLEDLQ

SEQ ID NO: 32 - protein, 14447 aa, Homo sapiens
DKTLASPTSSVVGRTTQSLGVMSSALPESTSRGMTHSEQRTSPSLSPQVNGTPSRNYPATSMVSGLSSPRTRTSSTEGNFTKEASTYTLTVETTSGPVTEKYTVPTETSTTEGDSTETPWDTRYIPVKITSPMKTFADSTASKENAPVSMTPAETTVTDSHTPGRTNPSFGTLYSSFLDLSPKGTPNSRGETSLELILSTTGYPFSSPEPGSAGHSRISTSAPLSSSASVLDNKISETSIFSGQSLTSPLSPGVPEARASTMPNSAIPFSMTLSNAETSAERVRSTISSLGTPSISTKQTAETILTFHAFAETMDIPSTHIAKTLASEWLGSPGTLGGTSTSALTTTSPSTTLVSEETNTHHSTSGKETEGTLNTSMTPLETSAPGEESEMTATLVPTLGFTTLDSKIRSPSQVSSSHPTRELRTTGSTSGRQSSSTAAHGSSDILRATTSSTSKASSWTSESTAQQFSEPQHTQWVETSPSMKTERPPASTSVAAPITTSVPSVVSGFTTLKTSSTKGIWLEETSADTLIGESTAGPTTHQFAVPTGISMTGGSSTRGSQGTTHLLTRATASSETSADLTLATNGVPVSVSPAVSKTAAGSSPPGGTKPSYTMVSSVIPETSSLQSSAFREGTSLGLTPLNTRHPFSSPEPDSAGHTKISTSIPLLSSASVLEDKVSATSTFSHHKATSSITTGTPEISTKTKPSSAVLSSMTLSNAATSPERVRNATSPLTHPSPSGEETAGSVLTLSTSAETTDSPNIHPTGTLTSESSESPSTLSLPSVSGVKTTFSSSTPSTHLFTSGEETEETSNPSVSQPETSVSRVRTTLASTSVPTPVFPTMDTWPTRSAQFSSSHLVSELRATSSTSVTNSTGSALPKISHLTGTATMSQTNRDTFNDSAAPQSTTWPETSPRFKTGLPSATTTVSTSATSLSATVMVSKFTSPATSSMEATSIREPSTTILTTETTNGPGSMAVASTNIPIGKGYITEGRLDTSHLPIGTTASSETSMDFTMAKESVSMSVSPSQSMDAAGSSTPGRTSQFVDTFSDDVYHLTSREITIPRDGTSSALTPQMTATHPPSPDPGSARSTWLGILSSSPSSPTPKVTMSSTFSTQRVTTSMIMDTVETSRWNMPNLPSTTSLTPSNIPTSGAIGKSTLVPLDTPSPATSLEASEGGLPTLSTYPESTNTPSIHLGAHASSESPSTIKLTMASVVKPGSYTPLTFPSIETHIHVSTARMAYSSGSSPEMTAPGETNTGSTWDPTTYITTTDPKDTSSAQVSTPHSVRTLRTTENHPKTESATPAAYSGSPKISSSPNLTSPATKAWTITDTTEHSTQLHYTKLAEKSSGFETQSAPGPVSVVIPTSPTIGSSTLELTSDVPGEPLVLAPSEQTTITLPMATWLSTSLTEEMASTDLDISSPSSPMSTFAIFPPMSTPSHELSKSEADTSAIRNTDSTTLDQHLGIRSLGRTGDLTTVPITPLTTTWTSVIEHSTQAQDTLSATMSPTHVTQSLKDQTSIPASASPSHLTEVYPELGTQGRSSSEATTFWKPSTDTLSREIETGPTNIQSTPPMDNTTTGSSSSGVTLGIAHLPIGTSSPAETSTNMALERRSSTATVSMAGTMGLLVTSAPGRSISQSLGRVSSVLSESTTEGVTDSSKGSSPRLNTQGNTALSSSLEPSYAEGSQMSTSIPLTSSPTTPDVEFIGGSTFWTKEVTTVMTSDISKSSARTESSSATLMSTALGSTENTGKEKLRTASMDLPSPTPSMEVTPWISLTLSNAPNTTDSLDLSHGVHTSSAGTLATDRSLNTGVTRASRLENGSDTSSKSLSMGNSTHTSMTYTEKSEVSSSIHPRPETSAPGAETTLTSTPGNRAISLTLPFSSIPVEEVISTGITSGPDINSAPMTHSPITPPTIVWTSTGTIEQSTQPLHAVSSEKVSVQTQSTPYVNSVAVSASPTHENSVSSGSSTSSPYSSASLESLDSTISRRNAITSWLWDLTTSLPTTTWPSTSLSEALSSGHSGVSNPSSTTTEFPLFSAASTSAAKQRNPETETHGPQNTAASTLNTDASSVTGLSETPVGASISSEVPLPMAITSRSDVSGLTSESTANPSLGTASSAGTKLTRTISLPTSESLVSFRMNKDPWTVSIPLGSHPTTNTETSIPVNSAGPPGLSTVASDVIDTPSDGAESIPTVSFSPSPDTEVTTISHFPEKTTHSFRTISSLTHELTSRVTPIPGDWMSSAMSTKPTGASPSITLGERRTITSAAPTTSPIVLTASFTETSTVSLDNETTVKTSDILDARKTNELPSDSSSSSDLINTSIASSTMDVTKTASISPTSISGMTASSSPSLFSSDRPQVPTSTTETNTATSPSVSSNTYSLDGGSNVGGTPSTLPPFTITHPVETSSALLAWSRPVRTFSTMVSTDTASGENPTSSNSVVTSVPAPGTWTSVGSTTDLPAMGFLKTSPAGEAHSLLASTIEPATAFTPHLSAAVVTGSSATSEASLLTTSESKAIHSSPQTPTTPTSGANWETSATPESLLVVTETSDTTLTSKILVTDTILFSTVSTPPSKFPSTGTLSGASFPTLLPDTPAIPLTATEPTSSLATSFDSTPLVTIASDSLGTVPETTLTMSETSNGDALVLKTVSNPDRSIPGITIQGVTESPLHPSSTSPSKIVAPRNTTYEGSITVALSTLPAGTTGSLVFSQSSENSETTALVDSSAGLERASVMPLTTGSQGMASSGGIRSGSTHSTGTKTFSSLPLTMNPGEVTAMSEITTNRLTATQSTAPKGIPVKPTSAESGLLTPVSASSSPSKAFASLTTAPPTWGIPQSTLTFEFSEVPSLDTKSASLPTPGQSLNTIPDSDASTASSSLSKSPEKNPRARMMTSTKAISASSFQSTGFTETPEGSASPSMAGHEPRVPTSGTGDPRYASESMSYPDPSKASSAMTSTSLASKLTTLFSTGQAARSGSSSSPISLSTEKETSFLSPTASTSRKTSLFLGPSMARQPNILVHLQTSALTLSPTSTLNMSQEEPPELTSSQTIAEEEGTTAETQTLTFTPSETPTSLLPVSSPTEPTARRKSSPETWASSISVPAKTSLVETTDGTLVTTIKMSSQAAQGNSTWPAPAEETGSSPAGTSPGSPEMSTTLKIMSSKEPSISPEIRSTVRNSPWKTPETTVPMETTVEPVTLQSTALGSGSTSISHLPTGTTSPTKSPTENMLATERVSLSPSPPEAWTNLYSGTPGGTRQSLATMSSVSLESPTARSITGTGQQSSPELVSKTTGMEFSMWHGSTGGTTGDTHVSLSTSSNILEDPVTSPNSVSSLTDKSKHKTETWVSTTAIPSTVLNNKIMAAEQQTSRSVDEAYSSTSSWSDQTSGSDITLGASPDVTNTLYITSTAQTTSLVSLPSGDQGITSLTNPSGGKTSSASSVTSPSIGLETLRANVSAVKSDIAPTAGHLSQTSSPAEVSILDVTTAPTPGISTTITTMGTNSISTTTPNPEVGMSTMDSTPATERRTTSTEHPSTWSSTAASDSWTVTDMTSNLKVARSPGTISTMHTTSFLASSTELDSMSTPHGRITVIGTSLVTPSSDASAVKTETSTSERTLSPSDTTASTPISTFSRVQRMSISVPDILSTSWTPSSTEAEDVPVSMVSTDHASTKTDPNTPLSTFLFDSLSTLDWDTGRSLSSATATTSAPQGATTPQELTLETMISPATSQLPFSIGHITSAVTPAAMARSSGVTFSRPDPTSKKAEQTSTQLPTTTSAHPGQVPRSAATTLDVIPHTAKTPDATFQRQGQTALTTEARATSDSWNEKEKSTPSAPWITEMMNSVSEDTIKEVTSSSSVLRTLNTLDINLESGTTSSPSWKSSPYERIAPSESTTDKEAIHPSTNTVETTGWVTSSEHASHSTIPAHSASSKLTSPVVTTSTREQAIVSMSTTTWPESTRARTEPNSFLTIELRDVSPYMDTSSTTQTSIISSPGSTAITKGPRTEITSSKRISSSFLAQSMRSSDSPSEAITRLSNFPAMTESGGMILAMQTSPPGATSLSAPTLDTSATASWTGTPLATTQRFTYSEKTTLFSKGPEDTSQPSPPSVEETSSSSSLVPIHATTSPSNILLTSQGHSPSSTPPVTSVFLSETSGLGKTTDMSRISLEPGTSLPPNLSSTAGEALSTYEASRDTKAIHHSADTAVTNMEATSSEYSPIPGHTKPSKATSPLVTSHIMGDITSSTSVFGSSETTEIETVSSVNQGLQERSTSQVASSATETSTVITHVSSGDATTHVTKTQATFSSGTSISSPHQFITSTNTFTDVSTNPSTSLIMTESSGVTITTQTGPTGAATQGPYLLDTSTMPYLTETPLAVTPDFMQSEKTTLISKGPKDVSWTSPPSVAETSYPSSLTPFLVTTIPPATSTLQGQHTSSPVSATSVLTSGLVKTTDMLNTSMEPVTNSPQNLNNPSNEILATLAATTDIETIHPSINKAVTNMGTASSAHVLHSTLPVSSEPSTATSPMVPASSMGDALASISIPGSETTDIEGEPTSSLTAGRKENSTLQEMNSTTESNIILSNVSVGAITEATKMEVPSFDATFIPTPAQSTKFPDIFSVASSRLSNSPPMTISTHMTTTQTGSSGATSKIPLALDTSTLETSAGTPSVVTEGFAHSKITTAMNNDVKDVSQTNPPFQDEASSPSSQAPVLVTTLPSSVAFTPQWHSTSSPVSMSSVLTSSLVKTAGKVDTSLETVTSSPQSMSNTLDDISVTSAATTDIETTHPSINTVVTNVGTTGSAFESHSTVSAYPEPSKVTSPNVTTSTMEDTTISRSIPKSSKTTRTETETTSSLTPKLRETSISQEITSSTETSTVPYKELTGATTEVSRTDVTSSSSTSFPGPDQSTVSLDISTETNTRLSTSPIMTESAEITITTQTGPHGATSQDTFTMDPSNTTPQAGIHSAMTHGFSQLDVTTLMSRIPQDVSWTSPPSVDKTSSPSSFLSSPAMTTPSLISSTLPEDKLSSPMTSLLTSGLVKITDILRTRLEPVTSSLPNFSSTSDKILATSKDSKDTKEIFPSINTEETNVKANNSGHESHSPALADSETPKATTQMVITTTVGDPAPSTSMPVHGSSETTNIKREPTYFLTPRLRETSTSQESSFPTDTSFLLSKVPTGTITEVSSTGVNSSSKISTPDHDKSTVPPDTFTGEIPRVFTSSIKTKSAEMTITTQASPPESASHSTLPLDTSTTLSQGGTHSTVTQGFPYSEVTTLMGMGPGNVSWMTTPPVEETSSVSSLMSSPAMTSPSPVSSTSPQSIPSSPLPVTALPTSVLVTTTDVLGTTSPESVTSSPPNLSSITHERPATYKDTAHTEAAMHHSTNTAVTNVGTSGSGHKSQSSVLADSETSKATPLMSTTSTLGDTSVSTSTPNISQTNQIQTEPTASLSPRLRESSTSEKTSSTTETNTAFSYVPTGAITQASRTEISSSRTSISDLDRPTIAPDISTGMITRLFTSPIMTKSAEMTVTTQTTTPGATSQGILPWDTSTTLFQGGTHSTVSQGFPHSEITTLRSRTPGDVSWMTTPPVEETSSGFSLMSPSMTSPSPVSSTSPESIPSSPLPVTALLTSVLVTTTNVLGTTSPEPVTSSPPNLSSPTQERLTTYKDTAHTEAMHASMHTNTAVANVGTSISGHESQSSVPADSHTSKATSPMGITFAMGDTSVSTSTPAFFETRIQTESTSSLIPGLRDTRTSEEINTVTETSTVLSEVPTTTTTEVSRTEVITSSRTTISGPDHSKMSPYISTETITRLSTFPFVTGSTEMAITNQTGPIGTISQATLTLDTSSTASWEGTHSPVTQRFPHSEETTTMSRSTKGVSWQSPPSVEETSSPSSPVPLPAITSHSSLYSAVSGSSPTSALPVTSLLTSGRRKTIDMLDTHSELVTSSLPSASSFSGEILTSEASTNTETIHFSENTAETNMGTTNSMHKLHSSVSIHSQPSGHTPPKVTGSMMEDAIVSTSTPGSPETKNVDRDSTSPLTPELKEDSTALVMNSTTESNTVFSSVSLDAATEVSRAEVTYYDPTFMPASAQSTKSPDISPEASSSHSNSPPLTISTHKTIATQTGPSGVTSLGQLTLDTSTIATSAGTPSARTQDFVDSETTSVMNNDLNDVLKTSPFSAEEANSLSSQAPLLVTTSPSPVTSTLQEHSTSSLVSVTSVPTPTLAKITDMDTNLEPVTRSPQNLRNTLATSEATTDTHTMHPSINTAVANVGTTSSPNEFYFTVSPDSDPYKATSAVVITSTSGDSIVSTSMPRSSAMKKIESETTFSLIFRLRETSTSQKIGSSSDTSTVFDKAFTAATTEVSRTELTSSSRTSIQGTEKPTMSPDTSTRSVTMLSTFAGLTKSEERTIATQTGPHRATSQGTLTWDTSITTSQAGTHSAMTHGFSQLDLSTLTSRVPEYISGTSPPSVEKTSSSSSLLSLPAITSPSPVPTTLPESRPSSPVHLTSLPTSGLVKTTDMLASVASLPPNLGSTSHKIPTTSEDIKDTEKMYPSTNIAVTNVGTTTSEKESYSSVPAYSEPPKVTSPMVTSFNIRDTIVSTSMPGSSEITRIEMESTFSLAHGLKGTSTSQDPIVSTEKSAVLHKLTTGATETSRTEVASSRRTSIPGPDHSTESPDISTEVIPSLPISLGITESSNMTIITRTGPPLGSTSQGTFTLDTPTTSSRAGTHSMATQEFPHSEMTTVMNKDPEILSWTIPPSIEKTSFSSSLMPSPAMTSPPVSSTLPKTIHTTPSPMTSLLTPSLVMTTDTLGTSPEPTTSSPPNLSSTSHEILTTDEDTTAIEAMHPSTSTAATNVETTSSGHGSQSSVLADSEKTKATAPMDTTSTMGHTTVSTSMSVSSETTKIKRESTYSLTPGLRETSISQNASFSTDTSIVLSEVPTGTTAEVSRTEVTSSGRTSIPGPSQSTVLPEISTRTMTRLFASPTMTESAEMTIPTQTGPSGSTSQDTLTLDTSTTKSQAKTHSTLTQRFPHSEMTTLMSRGPGDMSWQSSPSLENPSSLPSLLSLPATTSPPPISSTLPVTISSSPLPVTSLLTSSPVTTTDMLHTSPELVTSSPPKLSHTSDERLTTGKDTTNTEAVHPSTNTAASNVEIPSSGHESPSSALADSETSKATSPMFITSTQEDTTVAISTPHFLETSRIQKESISSLSPKLRETGSSVETSSAIETSAVLSEVSIGATTEISRTEVTSSSRTSISGSAESTMLPEISTTRKIIKFPTSPILAESSEMTIKTQTSPPGSTSESTFTLDTSTTPSLVITHSTMTQRLPHSEITTLVSRGAGDVPRPSSLPVEETSPPSSQLSLSAMISPSPVSSTLPASSHSSSASVTSLLTPGQVKTTEVLDASAEPETSSPPSLSSTSVEILATSEVTTDTEKIHPFSNTAVTKVGTSSSGHESPSSVLPDSETTKATSAMGTISIMGDTSVSTLTPALSNTRKIQSEPASSLTTRLRETSTSEETSLATEANTVLSKVSTGATTEVSRTEAISFSRTSMSGPEQSTMSQDISIGTIPRISASSVLTESAKMTITTQTGPSESTLESTLNLNTATTPSWVETHSIVIQGFPHPEMTTSMGRGPGGVSWPSPPFVKETSPPSSPLSLPAVTSPHPVSTTFLAHIPPSPLPVTSLLTSGPATTTDILGTSTEPGTSSSSSLSTTSHERLTTYKDTAHTEAVHPSTNTGGTNVATTSSGYKSQSSVLADSSPMCTTSTMGDTSVLTSTPAFLETRRIQTELASSLTPGLRESSGSEGTSSGTKMSTVLSKVPTGATTEISKEDVTSIPGPAQSTISPDISTRTVSWFSTSPVMTESAEITMNTHTSPLGATTQGTSTLDTSSTTSLTMTHSTISQGFSHSQMSTLMRRGPEDVSWMSPPLLEKTRPSFSLMSSPATTSPSPVSSTLPESISSSPLPVTSLLTSGLAKTTDMLHKSSEPVTNSPANLSSTSVEILATSEVTTDTEKTHPSSNRTVTDVGTSSSGHESTSFVLADSQTSKVTSPMVITSTMEDTSVSTSTPGFFETSRIQTEPTSSLTLGLRKTSSSEGTSLATEMSTVLSGVPTGATAEVSRTEVTSSSRTSISGFAQLTVSPETSTETITRLPTSSIMTESAEMMIKTQTDPPGSTPESTHTVDISTTPNWVETHSTVTQRFSHSEMTTLVSRSPGDMLWPSQSSVEETSSASSLLSLPATTSPSPVSSTLVEDFPSASLPVTSLLNPGLVITTDRMGISREPGTSSTSNLSSTSHERLTTLEDTVDTEDMQPSTHTAVTNVRTSISGHESQSSVLSDSETPKATSPMGTTYTMGETSVSISTSDFFETSRIQIEPTSSLTSGLRETSSSERISSATEGSTVLSEVPSGATTEVSRTEVISSRGTSMSGPDQFTISPDISTEAITRLSTSPIMTESAESAITIETGSPGATSEGTLTLDTSTTTFWSGTHSTASPGFSHSEMTTLMSRTPGDVPWPSLPSVEEASSVSSSLSSPAMTSTSFFSTLPESISSSPHPVTALLTLGPVKTTDMLRTSSEPETSSPPNLSSTSAEILATSEVTKDREKIHPSSNTPVVNVGTVIYKHLSPSSVLADLVTTKPTSPMATTSTLGNTSVSTSTPAFPETMMTQPTSSLTSGLREISTSQETSSATERSASLSGMPTGATTKVSRTEALSLGRTSTPGPAQSTISPEISTETITRISTPLTTTGSAEMTITPKTGHSGASSQGTFTLDTSSRASWPGTHSAATHRSPHSGMTTPMSRGPEDVSWPSRPSVEKTSPPSSLVSLSAVTSPSPLYSTPSESSHSSPLRVTSLFTPVMMKTTDMLDTSLEPVTTSPPSMNITSDESLATSKATMETEAIQLSENTAVTQMGTISARQEFYSSYPGLPEPSKVTSPVVTSSTIKDIVSTTIPASSEITRIEMESTSTLTPTPRETSTSQEIHSATKPSTVPYKALTSATIEDSMTQVMSSSRGPSPDQSTMSQDISTEVITRLSTSPIKTESTEMTITTQTGSPGATSRGTLTLDTSTTFMSGTHSTASQGFSHSQMTALMSRTPGDVPWLSHPSVEEASSASFSLSSPVMTSSSPVSSTLPDSIHSSSLPVTSLLTSGLVKTTELLGTSSEPETSSPPNLSSTSAEILAITEVTTDTEKLEMTNVVTSGYTHESPSSVLADSVTTKATSSMGITYPTGDTNVLTSTPAFSDTSRIQTKSKLSLTPGLMETSISEETSSATEKSTVLSSVPTGATTEVSRTEAISSSRTSIPGPAQSTMSSDTSMETITRISTPLTRKESTDMAITPKTGPSGATSQGTFTLDSSSTASWPGTHSATTQRFPQSVVTTPMSRGPEDVSWPSPLSVEKNSPPSSLVSSSSVTSPSPLYSTPSGSSHSSPVPVTSLFTSIMMKATDMLDASLEPETTSAPNMNITSDESLAASKATTETEAIHVFENTAASHVETTSATEELYSSSPGFSEPTKVISPVVTSSSIRDNMVSTTMPGSSGITRIEIESMSSLTPGLRETRTSQDITSSTETSTVLYKMPSGATPEVSRTEVMPSSRTSIPGPAQSTMSLDISDEVVTRLSTSPIMTESAEITITTQTGYSLATSQVTLPLGTSMTFLSGTHSTMSQGLSHSEMTNLMSRGPESLSWTSPRFVETTRSSSSLTSLPLTTSLSPVSSTLLDSSPSSPLPVTSLILPGLVKTTEVLDTSSEPKTSSSPNLSSTSVEIPATSEIMTDTEKIHPSSNTAVAKVRTSSSVHESHSSVLADSETTITIPSMGITSAVDDTTVFTSNPAFSETRRIPTEPTFSLTPGFRETSTSEETTSITETSAVLYGVPTSATTEVSMTEIMSSNRIHIPDSDQSTMSPDIITEVITRLSSSSMMSESTQMTITTQKSSPGATAQSTLTLATTTAPLARTHSTVPPRFLHSEMTTLMSRSPENPSWKSSLFVEKTSSSSSLLSLPVTTSPSVSSTLPQSIPSSSFSVTSLLTPGMVKTTDTSTEPGTSLSPNLSGTSVEILAASEVTTDTEKIHPSSSMAVTNVGTTSSGHELYSSVSIHSEPSKATYPVGTPSSMAETSISTSMPANFETTGFEAEPFSHLTSGFRKTNMSLDTSSVTPTNTPSSPGSTHLLQSSKTDFTSSAKTSSPDWPPASQYTEIPVDIITPFNASPSITESTGITSFPESRFTMSVTESTHHLSTDLLPSAETISTGTVMPSLSEAMTSFATTGVPRAISGSGSPFSRTESGPGDATLSTIAESLPSSTPVPFSSSTFTTTDSSTIPALHEITSSSATPYRVDTSLGTESSTTEGRLVMVSTLDTSSQPGRTSSSPILDTRMTESVELGTVTSAYQVPSLSTRLTRTDGIMEHITKIPNEAAHRGTIRPVKGPQTSTSPASPKGLHTGGTKRMETTTTALKTTTTALKTTSRATLTTSVYTPTLGTLTPLNASMQMASTIPTEMMITTPYVFPDVPETTSSLATSLGAETSTALPRTTPSVFNRESETTASLVSRSGAERSPVIQTLDVSSSEPDTTASWVIHPAETIPTVSKTTPNFFHSELDTVSSTATSHGADVSSAIPTNISPSELDALTPLVTISGTDTSTTFPTLTKSPHETETRTTWLTHPAETSSTIPRTIPNFSHHESDATPSIATSPGAETSSAIPIMTVSPGAEDLVTSQVTSSGTDRNMTIPTLTLSPGEPKTIASLVTHPEAQTSSAIPTSTISPAVSRLVTSMVTSLAAKTSTTNRALTNSPGEPATTVSLVTHPAQTSPTVPWTTSIFFHSKSDTTPSMTTSHGAESSSAVPTPTVSTEVPGVVTPLVTSSRAVISTTIPILTLSPGEPETTPSMATSHGEEASSAIPTPTVSPGVPGVVTSLVTSSRAVTSTTIPILTFSLGEPETTPSMATSHGTEAGSAVPTVLPEVPGMVTSLVASSRAVTSTTLPTLTLSPGEPETTPSMATSHGAEASSTVPTVSPEVPGVVTSLVTSSSGVNSTSIPTLILSPGELETTPSMATSHGAEASSAVPTPTVSPGVSGVVTPLVTSSRAVTSTTIPILTLSSSEPETTPSMATSHGVEASSAVLTVSPEVPGMVTSLVTSSRAVTSTTIPTLTISSDEPETTTSLVTHSEAKMISAIPTLAVSPTVQGLVTSLVTSSGSETSAFSNLTVASSQPETIDSWVAHPGTEASSVVPTLTVSTGEPFTNISLVTHPAESSSTLPRTTSRFSHSELDTMPSTVTSPEAESSSAISTTISPGIPGVLTSLVTSSGRDISATFPTVPESPHESEATASWVTHPAVTSTTVPRTTPNYSHSEPDTTPSIATSPGAEATSDFPTITVSPDVPDMVTSQVTSSGTDTSITIPTLTLSSGEPETTTSFITYSETHTSSAIPTLPVSPGASKMLTSLVISSGTDSTTTFPTLTETPYEPETTAIQLIHPAETNTMVPRTTPKFSHSKSDTTLPVAITSPGPEASSAVSTTTISPDMSDLVTSLVPSSGTDTSTTFPTLSETPYEPETTATWLTHPAETSTTVSGTIPNFSHRGSDTAPSMVTSPGVDTRSGVPTTTIPPSIPGVVTSQVTSSATDTSTAIPTLTPSPGEPETTASSATHPGTQTGFTVPIRTVPSSEPDTMASWVTHPPQTSTPVSRTTSSFSHSSPDATPVMATSPRTEASSAVLTTISPGAPEMVTSQITSSGAATSTTVPTLTHSPGMPETTALLSTHPRTETSKTFPASTVFPQVSETTASLTIRPGAETSTALPTQTTSSLFTLLVTGTSRVDLSPTASPGVSAKTAPLSTHPGTETSTMIPTSTLSLGLLETTGLLATSSSAETSTSTLTLTVSPAVSGLSSASITTDKPQTVTSWNTETSPSVTSVGPPEFSRTVTGTTMTLIPSEMPTPPKTSHGEGVSPTTILRTTMVEATNLATTGSSPTVAKTTTTFNTLAGSLFTPLTTPGMSTLASESVTSRTSYNHRSWISTTSSYNRRYWTPATSTPVTSTFSPGISTSSIPSSTAATVPFMVPFTLNFTITNLQYEEDMRHPGSRKFNATERELQGLLKPLFRNSSLEYLYSGCRLASLRPEKDSSATAVDAICTHRPDPEDLGLDRERLYWELSNLTNGIQELGPYTLDRNSLYVNGFTHRSSMPTTSTPGTSTVDVGTSGTPSSSPSPTTAGPLLMPFTLNFTITNLQYEEDMRRTGSRKFNTMESVLQGLLKPLFKNTSVGPLYSGCRLTLLRPEKDGAATGVDAICTHRLDPKSPGLNREQLYWELSKLTNDIEELGPYTLDRNSLYVNGFTHQSSVSTTSTPGTSTVDLRTSGTPSSLSSPTIMAAGPLLVPFTLNFTITNLQYGEDMGHPGSRKFNTTERVLQGLLGPIFKNTSVGPLYSGCRLTSLRSEKDGAATGVDAICIHHLDPKSPGLNRERLYWELSQLTNGIKELGPYTLDRNSLYVNGFTHRTSVPTSSTPGTSTVDLGTSGTPFSLPSPATAGPLLVLFTLNFTITNLKYEEDMHRPGSRKFNTTERVLQTLLGPMFKNTSVGLLYSGCRLTLLRSEKDGAATGVDAICTHRLDPKSPGVDREQLYWELSQLTNGIKELGPYTLDRNSLYVNGFTHWIPVPTSSTPGTSTVDLGSGTPSSLPSPTTAGPLLVPFTLNFTITNLKYEEDMHCPGSRKFNTTERVLQSLLGPMFKNTSVGPLYSGCRLTLLRSEKDGAATGVDAICTHRLDPKSPGVDREQLYWELSQLTNGIKELGPYTLDRNSLYVNGFTHQTSAPNTSTPGTSTVDLGTSGTPSSLPSPTSAGPLLVPFTLNFTITNLQYEEDMHHPGSRKFNTTERVLQGLLGPMFKNTSVGLLYSGCRLTLLRPEKNGAATGMDAICSHRLDPKSPGLNREQLYWELSQLTHGIKELGPYTLDRNSLYVNGFTHRSSVAPTSTPGTSTVDLGTSGTPSSLPSPTTAVPLLVPFTLNFTITNLQYGEDMRHPGSRKFNTTERVLQGLLGPLFKNSSVGPLYSGCRLISLRSEKDGAATGVDAICTHHLNPQSPGLDREQLYWQLSQMTNGIKELGPYTLDRNSLYVNGFTHRSSGLTTSTPWTSTVDLGTSGTPSPVPSPTTTGPLLVPFTLNFTITNLQYEENMGHPGSRKFNITESVLQGLLKPLFKSTSVGPLYSGCRLTLLRPEKDGVATRVDAICTHRPDPKIPGLDRQQLYWELSQLTHSITELGPYTLDRDSLYVNGFTQRSSVPTTSTPGTFTVQPETSETPSSLPGPTATGPVLLPFTLNFTITNLQYEEDMRRPGSRKFNTTERVLQGLLMPLFKNTSVSSLYSGCRLTLLRPEKDGAATRVDAVCTHRPDPKSPGLDRERLYWKLSQLTHGITELGPYTLDRHSLYVNGFTHQSSMTTTRTPDTSTMHLATSRTPASLSGPMTASPLLVLFTINFTITNLRYEENMHHPGSRKFNTTERVLQGLLRPVFKNTSVGPLYSGCRLTLLRPKKDGAATKVDAICTYRPDPKSPGLDREQLYWELSQLTHSITELGPYTLDRDSLYVNGFTQRSSVPTTSIPGTPTVDLGTSGTPVSKPGPSAASPLLVLFTLNFTITNLRYEENMQHPGSRKFNTTERVLQGLLRSLFKSTSVGPLYSGCRLTLLRPEKDGTATGVDAICTHHPDPKSPRLDREQLYWELSQLTHNITELGPYALDNDSLFVNGFTHRSSVSTTSTPGTPTVYLGASKTPASIFGPSAASHLLILFTLNFTITNLRYEENMWPGSRKFNTTERVLQGLLRPLFKNTSVGPLYSGCRLTLLRPEKDGEATGVDAICTHRPDPTGPGLDREQLYLELSQLTHSITELGPYTLDRDSLYVNGFTHRSSVPTTSTGVVSEEPFTLNFTINNLRYMADMGQPGSLKFNITDNVMQHLLSPLFQRSSLGARYTGCRVIALRSVKNGAETRVDLLCTYLQPLSGPGLPIKQVFHELSQQTHGITRLGPYSLDKDSLYLNGYNEPGPDEPPTTPKPATTFLPPLSEATTAMGYHLKTLTLNFTISNLQYSPDMGKGSATFNSTEGVLQHLLRPLFQKSSMGPFYLGCQLISLRPEKDGAATGVDTTCTYHPDPVGPGLDIQQLYWELSQLTHGVTQLGFYVLDRDSLFINGYAPQNLSIRGEYQINFHIVNWNLSNPDPTSSEYITLLRDIQDKVTTLYKGSQLHDTFRFCLVTNLTMDSVLVTVKALFSSNLDPSLVEQVFLDKTLNASFHWLGSTYQLVDIHVTEMESSVYQPTSSSSTQHFYLNFTITNLPYSQDKAQPGTTNYQRNKRNIEDALNQLFRNSSIKSYFSDCQVSTFRSVPNRHHTGVDSLCNFSPLARRVDRVAIYEEFLRMTRNGTQLQNFTLDRSSVLVDGYSPNRNEPLTGNSDLPFWAVILIGLAGLLGVITCLICGVLVTTRRRKKEGEYNVQQQCPGYYQSHLDLEDLQ

SEQ ID NO: 33 - protein, 6 aa, synthetic construct
  REGION 1..6: note = Description of Artificial Sequence: Synthetic 6xHis tag
HHHHHH